European Patent Specification EP 3 347 043 B1, published January 7, 2026. Title: PROCESS FOR PREPARING AN ATTENUATED TETRAVALENT DENGUE VACCINE. Applicant: Frazatti Gallina, Neuza M. The sequence listing filed with the application follows.

SEQUENCE LISTING (4 sequences)

SEQ ID NO: 1 - DNA, 10703 bp, Dengue virus 1
  misc_feature (1)..(7): n is a, c, g, or t
nnnnnnnagtctacgtggaccgacaagaacagtttcgaatcggaagcttgcttaacgtagttctaacagttttttattagagagcagatctctgatgaacaaccaacggaaaaagacgggtcgaccgtctttcaatatgctgaaacgcgcgagaaaccgcgtgtcaactgtttcacagttggcgaagagattctcaaaaggattgctttcaggccaaggacccatgaaattggtgatggcttttatagcattcctaagatttctagccatacctccaacagcaggaattttggctagatggggctcattcaagaagaatggagcgatcaaagtgttacggggtttcaagaaagaaatctcaaacatgttgaacataatgaacaggaggaaaagatctgtgaccatgctcctcatgctgctgcccacagccctggcgttccatctgaccacccgagggggagagccgcacatgatagttagcaagcaggaaagaggaaaatcacttttgtttaagacctctgcaggtgtcaacatgtgcacccttattgcaatggatttgggagagttatgtgaggacacaatgacctacaaatgcccccggatcactgagacggaaccagatgacgttgactgttggtgcaatgccacggagacatgggtgacctatggaacatgttctcaaactggtgaacaccgacgagacaaacgttccgtcgcactggcaccacacgtagggcttggtctagaaacaagaaccgaaacgtggatgtcctctgaaggcgcttggaaacaaatacaaaaagtggagacctgggctctgagacacccaggattcacggtgatagccctttttctagcacatgccataggaacatccatcacccagaaagggatcatttttattttgctgatgctggtaactccatccatggccatgcggtgcgtgggaataggcaacagagacttcgtggaaggactgtcaggagctacgtgggtggatgtggtactggagcatggaagttgcgtcactaccatggcaaaagacaaaccaacactggacattgaactcttgaagacggaggtcacaaaccctgccgtcctgcgcaaactgtgcattgaagctaaaatatcaaacaccaccaccgattcgagatgtccaacacaaggagaagccacgctggtggaagaacaggacacgaactttgtgtgtcgacgaacgttcgtggacagaggctggggcaatggttgtgggctattcggaaaaggtagcttaataacgtgtgctaagtttaagtgtgtgacaaaactggaaggaaagatagtccaatatgaaaacttaaaatattcagtgatagtcaccgtacacactggagaccagcaccaagttggaaatgagaccacagaacatggaacaactgcaaccataacacctcaagctcccacgtcggaaatacagctgacagactacggagctctaacattggattgttcacctagaacagggctagactttaatgagatggtgttgttgacaatggaaaaacgatcgtggctcgtccacaaacaatggtttctagacttaccactgccttggacctcgggggcttcaacatcccaagagacttggaatagacaagacttgctggtcacatttaagacagctcatgcaaaaaagcaggaagtagtcgtactaggatcacaagaaggagcaatgcacactgcgttgactggagcgacagaaatccaaacgtctggaacgacaacaatttttgcaggacacctgaaatgcagactaaaaatggataaactgactttaaaagggatgtcatatgtaatgtgcacagggtcattcaagttagagaaggaagtggctgagacccagcatggaactgttctagtgcaggttaaatacgaaggaacagatgcaccatgcaagatccccttctcgtcccaagatgagaagggagtaacccagaatgggagattgataacagccaaccccatagtcactgacaaagaaaaaccagtcaacattgaagcggagccaccttttggtgagagctacattgtggtaggagcaggtgaaaaagctttgaaactaagctggttcaagaagggaagcagtatagggaaaatgtttgaagcaactgcccgtggagcacgaaggatggccatcctgggagacactgcatgggacttcggttctataggaggggtgttcacgtctgtgggaaaactgatacaccagatttttgggactgcgtatggagttttgttcagcggtgtttcttggaccatgaagataggaatagggattctgctgacatggctaggattaaactcaaggagcacgtccctttcaatgacgtgtatcgcagttggcatggtcacactgtacctaggagtcatggttcaggcggactcgggatgtgtaatcaactggaaaggcagagaactcaaatgtggaagcggcatttttgtcaccaatgaagtccacacctggacagagcaatataaattccaggccgactcccctaagagactatcagcggccattgggaaggcatgggaggagggtgtgtgtggaattcgatcagccactcgtctcgagaacatcatgtggaagcaaatatcaaatgaattaaaccacatcttacttgaaaatgacatgaaatttacagtggtcgtaggagacgttagtggaatcttggcccaaggaaagaaaatgattaggccacaacccatggaacacaaatactcgtggaaaagctggggaaaagccaaaatcataggagcagatgtacagaataccaccttcatcatcgacggcccaaacaccccagaatgccctgataaccaaagagcatggaacatttgggaagttgaagactatggatttggaattttcacgacaaacatatggttgaaattgcgtgactcctacactcaagtgtgtgaccaccggctaatgtcagctgccatcaaggatagcaaagcagtccatgctgacatggggtactggatagaaagtgaaaagaacgagacttggaagttggcaagagcctccttcatagaagttaagacatgcatctggccaaaatcccacactctatggagcaatggagtcctggaaagtgagatgataatcccaaagatatatggaggaccaatatctcagcacaactacagaccaggatatttcacacaaacagcagggccgtggcacttgggcaagttagaactagattttgatttatgtgaaggtaccactgttgttgtggatgaacattgtggaaatcgaggaccatctcttagaaccacaacagtcacaggaaagacaatccatgaatggtgctgtagatcttgcacgttaccccccctacgtttcaaaggagaagacgggtgctggtacggcatggaaatcagaccagtcaaggagaaggaagagaacctagttaagtcaatggtctctgcagggtcaggagaagtggacagtttttcactaggactgctatgcatatcaataatgatcgaagaggtaatgagatccagatggagcagaaaaatgctgatgactggaacattggctgtgttcctccttctcacaatgggacaattgacatggaatgatctgatcaggctatgtatcatggttggagccaacgcttcagacaagatggggatgggaacaacgtacctagctttgatggccactttcagaatgagaccaatgttcgcagtcgggctactgtttcgcagattaacatctagagaagttcttcttcttacagttggattgagtctggtggcatctgtagaactaccaaattccttagaggagctaggggatggacttgcaatgggcatcatgatgttgaaattactgactgattttcagtcacatcagctatgggctaccttgctgtctttaacatttgtcaaaacaactttttcattgcactatgcatggaagacaatggctatgatactgtcaattgtatctctcttccctttatgcctgtccacgacttctcaaaaaacaacatggcttccggtgttgctgggatctcttggatgcaaaccactaaccatgtttcttataacagaaaacaaaatctggggaaggaaaagctggcctctcaatgaaggaattatggctgttggaatagttagcattcttctaagttcacttctcaagaatgatgtgccactagctggcccactaatagctggaggcatgctaatagcatgttatgtcatatctggaagctcggccgatttatcactggagaaagcggctgaggtctcctgggaagaagaagcagaacactctggtgcctcacacaacatactagtggaggtccaagatgatggaaccatgaaaataaaggatgaagagagagatgacacactcaccattctcctcaaagcaactctgctagcaatctcaggggtatacccaatgtcaataccggcgaccctctttgtgtggtatttttggcagaaaaagaaacagagatcaggagtgctatgggacacacccagccctccagaagtggaaagagcagtccttgatgatggcatttatagaattctccaaagaggattgttgggcaggtctcaagtgggagtaggagtttttcaagaaggcgtgttccacacaatgtggcacgtcaccaggggagctgtcctcatgtaccaagggaagagactggaaccaagttgggccagtgtcaaaaaagacttgatctcatatggaggaggttggaggtttcaaggatcctggaacgcgggagaagaagtgcaggtgattgctgttgaaccggggaagaaccccaaaaatgtacagacagcgccgggtaccttcaagacccctgaaggcgaagttggagccatagctctagactttaaacccggcacatctggatctcctatcgtgaacagagagggaaaaatagtaggtctttatggaaatggagtggtgacaacaagtggtacctacgtcagtgccatagctcaagctaaagcatcacaagaagggcctctaccagagattgaggacgaggtgtttaggaaaagaaacttaacaataatggacctacatccaggatcgggaaaaacaagaagataccttccagccatagtccgtgaggccataaaaagaaagctgcgcacgctagtcttagctcccacaagagttgtcgcttctgaaatggcagaggcgctcaagggaatgccaataaggtatcagacaacagcagtgaagagtgaacacacgggaaaggagatagttgaccttatgtgtcacgccactttcactatgcgtctcctgtctcctgtgagagttcccaattataatatgattatcatggatgaagcacatttcaccgatccagccagcatagcagccagagggtatatctcaacccgagtgggtatgggtgaagcagctgcgattttcatgacagccactccccccggatcggtggaggcctttccacagagcaatgcagttatccaagatgaggaaagagacattcctgaaagatcatggaactcaggctatgactggatcactgatttcccaggtaaaacagtctggtttgttccaagcatcaaatcaggaaatgacattgccaactgtttaagaaagaatgggaaacgggtggtccaattgagcagaaaaacttttgacactgagtaccagaaaacaaaaaataacgactgggactatgttgtcacaacagacatatccgaaatgggagcaaacttccgagccgacagggtaatagacccgaggcggtgcctgaaaccggtaatactaaaagatggcccagagcgtgtcattctagccggaccgatgccagtgactgtggctagcgccgcccagaggagaggaagaattggaaggaaccaaaataaggaaggcgatcagtatatttacatgggacagcctctaaaaaatgatgaggaccacgcccattggacagaagcaaaaatgctccttgacaacataaacacaccagaagggattatcccagccctctttgagccggagagagaaaagagtgcagcaatagacggggaatacagactacggggtgaagcgaggaaaacgttcgtggagctcatgagaagaggagatctacctgtctggctatcctacaaagttgcctcagaaggcttccagtactccgacagaaggtggtgctttgatggggaaaggaacaaccaggtgttggaggagaacatggacgtggagatctggacaaaagaaggagaaagaaagaaactacgaccccgctggctggatgccagaacatactctgacccactggctctgcgcgaattcaaagagttcgcagcaggaagaagaagcgtctcaggtgacctaatattagaaatagggaaacttccacaacatttaacgcaaagggcccagaacgccttggacaatctggttatgttgcacaactctgaacaaggaggaaaagcctatagacacgccatggaagaactaccagacaccatagaaacgttaatgctcctagctttgatagctgtgctgactggtggagtgacgttgttcttcctatcaggaaggggtctaggaaaaacatccattggcctactctgcgtgattgcctcaagtgcactgttatggatggccagtgtggaaccccattggatagcggcctctatcatactggagttctttctgatggtgttgcttattccagagccggacagacagcgcactccacaagacaaccagctagcatacgtggtgataggtctgttattcatgatattgacagtggcagccaatgagatgggattactggaaaccacaaagaaggacctggggattggtcatgcagctgctgaaaaccaccatcatgctgcaatgctggacgtagacctacatccagcttcagcctggactctctacgcagtggccacaacaattatcactcccatgatgagacacacaattgaaaacacaacggcaaatatttccctgacagctattgcaaaccaggcagctatattgatgggacttgacaagggatggccaatatcaaagatggacataggagttccacttctcgccttggggtgctattctcaggtgaacccgctgacgctgacagcggcggtatttatgctagtggctcattatgccataattggacccggactgcaagcaaaagctactagagaagctcaaaaaaggacagcagccggaataatgaaaaacccaactgtcgacgggatcgttgcaatagatttggaccctgtggtttacgatgcaaaatttgaaaaacagctaggccaaataatgttgttgatactttgcacatcacagatcctcctgatgcggaccacatgggccttgtgtgaatccatcacactagccactggacctctgaccacgctttgggagggatctccaggaaaattctggaacaccacgatagcggtgtccatggcaaacatttttaggggaagttatctagcaggagcaggtctggccttttcattaatgaaatctctaggaggaggtaggagaggcacgggagcccaaggggaaacactgggagaaaaatggaaaagacagctaaaccaattgagcaagtcagaattcaacacttacaaaaggagtgggattatagaggtggatagatctgaagccaaagaggggttaaaaagaggagaaacgactaaacacgcagtgtcgagaggaacggccaaactgaggtggtttgtggagaggaaccttgtgaaaccagaagggaaagtcatagacctcggttgtggaagaggtggctggtcatattattgcgctgggctgaagaaagtcacagaagtgaaaggatacacgaaaggaggacctggacatgaggaaccaatcccaatggcaacctatggatggaacctagtaaagctatactccgggaaagatgtattctttacaccacctgagaaatgtgacaccctcttgtgtgatattggtgagtcctctccgaacccaactatagaagaaggaagaacgttacgtgttctaaagatggtggaaccatggctcagaggaaaccaattttgcataaaaattctaaatccctatatgccgagtgtggtagaaactttggagcaaatgcaaagaaaacatggaggaatgctagtgcgaaatccactctcaagaaactccactcatgaaatgtactgggtttcatgtggaacaggaaacattgtgtcagcagtaaacatgacatctagaatgctgctaaatcgattcacaatggctcacaggaagccaacatatgaaagagacgtggacttaggcgctggaacaagacatgtggcagtagaaccagaggtggccaacctagatatcattggccagaggatagagaatataaaaaatgaacacaaatcaacatggcattatgatgaggacaatccatacaaaacatgggcctatcatggatcatatgaggtcaagccatcaggatcagcctcatccatggtcaatggtgtggtgagactgctaaccaaaccatgggatgtcattcccatggtcacacaaatagccatgactgacaccacaccctttggacaacagagggtgtttaaagagaaagttgacacgcgtacaccaaaagcgaaacgaggcacagcacaaattatggaggtgacagccaggtggttatggggttttctctctagaaacaaaaaacccagaatctgcacaagagaggagttcacaagaaaagtcaggtcaaacgcagctattggagcagtgttcgttgatgaaaatcaatggaactcagcaaaagaggcagtggaagatgaacggttctgggaccttgtgcacagagagagggagcttcataaacaaggaaaatgtgccacgtgtgtctacaacatgatgggaaagagagagaaaaaattaggagagttcggaaaggcaaaaggaagtcgcgcaatatggtacatgtggttgggagcgcgctttttagagtttgaagcccttggtttcatgaatgaagatcactggttcagcagagagaattcactcagtggagtggaaggagaaggactccacaaacttggatacatactcagagacatatcaaagattccagggggaaatatgtatgcagatgacacagccggatgggacacaagaataacagaggatgatcttcagaatgaggccaaaatcactgacatcatggaacctgaacatgccctattggccacgtcaatctttaagctaacctaccaaaacaaggtagtaagggtgcagagaccagcgaaaaatggaaccgtgatggatgtcatatccagacgtgaccagagaggaagtggacaggttggaacctatggcttaaacaccttcaccaacatggaggcccaactaataagacaaatggagtctgagggaatcttttcacccagcgaattggaaaccccaaatctagccgaaagagtcctcgactggttgaaaaaacatggcaccgagaggctgaaaagaatggcaatcagtggagatgactgtgtggtgaaaccaattgatgacagatttgcaacagccttaacagctttgaatgacatgggaaaggtaagaaaagacataccgcaatgggaaccttcaaaaggatggaatgattggcaacaagtgcctttctgttcacaccatttccaccagctgattatgaaggatgggagggagatagtggtgccatgccgcaaccaagatgaacttgtaggtagggccagagtatcacaaggcgccggatggagcttgagagaaactgcatgcctaggcaagtcatatgcacaaatgtggcagctgatgtacttccacaggagagacttgagattagcggctaatgctatctgttcagccgttccagttgattgggtcccaaccagccgtaccacctggtcgatccatgcccaccatcaatggatgacaacagaagacatgttgtcagtgtggaatagggtttggatagaggaaaacccatggatggaggacaagactcatgtgtccagttgggaagacgttccatacctaggaaaaagggaagatcaatggtgtggatccctaataggcttaacagcacgagccacctgggccaccaacatacaagtggccataaaccaagtgagaaggctcattgggaatgagaattatctagacttcatgacatcaatgaagagattcaaaaacgagagtgatcccgaaggggcactctggtaagccaactcattcacaaaataaaggaaaataaaaaatcaaacaaggcaagaagtcaggccggattaagccatagcacggtaagagctatgctgcctgtgagccccgtccaaggacgtaaaatgaagtcaggccgaaagccacggttcgagcaagccgtgctgcctgtagctccatcgtggggatgtaaaaacccgggaggctgcaaaccatggaagctgtacgcatggggtagcagactagtggttagaggagacccctcccaagacacaacgcagcagcggggcccaagactagaggttagaggagaccccccgcacaacaacaaacagcatattgacgctgggagagaccagagatcctgctgtctctacagcatcattccaggcacagaacgccagaaaatggaatggtgctgttgaatcaacaggtt

SEQ ID NO: 2 - DNA, 10618 bp, Dengue virus 2
  misc_feature (1)..(23): n is a, c, g, or t
  misc_feature (10580)..(10618): n is a, c, g, or t
nnnnnnnnnnnnnnnnnnnnnnncaaggacagttccaaatcggaagcttgcttaacacagttctaacagtttgtttgaatagagagcagatctctggaaaaatgaaccaacgaaaaaaggtggttagaccacctttcaatatgctgaaacgcgagagaaaccgcgtatcaacccctcaagggctggtgaagagattctcaaccggacttttttctgggaaaggacccttacggatggtgctagcattcatcacgtttttgcgagtcctttccatcccaccaacagcagggattctgaagagatggggacagttgaagaaaaataaggccatcaagatactgattggattcaggaaggagataggccgcatgctgaacatcttgaacgggagaaaaaggtctgcaggcatgatcattatgctgattccaacagtgatggcgttccatttaaccacacgtaacggagaaccacacatgatcgtcagtagacaagagaaagggaaaagtcttctgtttaaaacagaggatggtgtgaacatgtgtaccctcatggccatggaccttggtgaattgtgtgaagatacaatcacgtacaagtgtcctcttctcaggcagaatgaaccagaagacatagattgttggtgcaactctacgtccacatgggtaacttatgggacgtgtaccaccacaggagaacacagaagagaaaaaagatcagtggcactcgttccacatgtgggaatgggactggagacacgaactgaaacatggatgtcatcagaaggggcctggaaacatgcccagagaattgaaacttggatcttgagacatccaggctttaccataatggcagcaatcctggcatacaccataggaacgacacatttccaaagagccctgattttcatcttactgacagctgtcgctccttcaatgacaatgcgttgcataggaatatcaaatagagactttgtagaaggggtttcaggaggaagctgggttgacatagtcttagaacatggaagctgtgtgacgacgatggcaaaaaacaaaccaacattggattttgaactgataaaaacagaagccaaacaacctgccactctaaggaagtactgtatagaggcaaagctgaccaacacaacaacagaatctcgctgcccaacacaaggagaacctagcctaaatgaagagcaggacaaaaggttcgtctgcaaacactccatggtggacagaggatggggaaatggatgtggattatttggaaaaggaggcattgtgacctgtgctatgttcacatgcaaaaagaacatggaaggaaaagtcgtgcaaccagaaaacttggaatacaccattgtgataacacctcactcaggggaagagcatgcagtcggaaatgacacaggaaaacatggcaaggaaatcaaaataacaccacagagttccatcacagaagcagagttgacaggctatggcactgtcacgatggaatgctttccgagaacgggcctcgacttcaatgagatggtgttgctgcaaatggaaaataaagcttggctggtgcacaggcaatggttcctagacctgccgttgccatggctgcccggagcggacacacaaggatcaaattggatacagaaagagacattggtcactttcaaaaatccccatgcgaagaaacaggatgttgttgttttgggatcccaagaaggggccatgcacacagcactcacaggggccacagaaatccagatgtcatcaggaaacttactgttcacaggacatctcaagtgcaggctgaggatggacaaactacagctcaaaggaatgtcatactctatgtgcacaggaaagtttaaagttgtgaaggaaatagcagaaacacaacatggaacaatagttatcagagtacaatatgaaggggacggttctccatgtaagatcccttttgagataatggatttggaaaaaagacatgttttaggtcgcctgattacagtcaacccaatcgtaacagaaaaagatagcccagtcaacatagaagcagaacctccattcggagacagctacatcatcataggagtagagccgggacaattgaagctcaactggtttaagaaaggaagttctatcggccaaatgtttgagacaacaatgaggggagcgaagagaatggccattttaggtgacacagcttgggattttggatccctgggaggagtgtttacatctataggaaaggctctccaccaagttttcggagcaatctatggggctgccttcagtggggtctcatggactatgaaaatcctcataggagtcattatcacatggataggaatgaactcgaggaacacttcaatggctatgacgtgcatagctgttggaggaatcactctgtttctgggcttcacagttcaagcagacatgggttgtgtggcgtcatggagtgggaaagaattgaagtgtggaagcggaatttttgtggttgacaacgtgcacacttggacagaacagtacaaatttcaaccagagtccccagcgagactagcgtctgcaatattaaatgcccacaaagatggggtctgtggaattagatcaaccacgaggctggaaaatgtcatgtggaagcaaataaccaacgagctaaactatgttctctgggaaggaggacatgacctcactgtagtggctggggatgtgaagggggtgttgaccaaaggcaagagagcactcacacccccagtgagtgatctgaaatattcatggaagacatggggaaaagcaaaaatcttcaccccagaagcaagaaatagcacatttttaatagacggaccagacacctctgaatgccccaatgaacgaagagcatggaactctcttgaggtggaagactatggatttggcatgttcacgaccaacatatggatgaaattccgagaaggaagttcagaagtgtgtgaccacaggttaatgtcagctgcaattaaagatcagaaagctgtgcatgctgacatgggttattggatagagagctcaaaaaaccagacctggcagatagagaaagcatctcttattgaagtgaaaacatgtctgtggcccaagacccacacactgtggagcaatggagtgctggaaagccagatgctcattccaaaatcatatgcgggccctttttcacagcacaattaccgccagggctatgccacgcaaaccgtgggcccatggcacttaggcaaattagagatagactttggagaatgccccggaacaacagtcacaattcaggaggattgtgaccatagaggcccatctttgaggaccaccactgcatctggaaaactagtcacgcaatggtgctgccgctcctgcacgatgcctcccttaaggttcttgggagaagatgggtgctggtatgggatggagattaggcccttgagtgaaaaagaagagaacatggtcaaatcacaggtgacggccggacagggcacatcagaaactttttctatgggtctgttgtgcctgaccttgtttgtggaagaatgcttgaggagaagagtcactaggaaacacatgatattagttgtggtgatcactctttgtgctatcatcctgggaggcctcacatggatggacttactacgagccctcatcatgttgggggacaccatgtctggtagaataggaggacagatccacctagccatcatggcagtgttcaagatgtcaccaggatacgtgctgggtgtgtttttaaggaaactcacttcaagagagacagcactaatggtaataggaatggccatgacaacggtgctttcaattccacatgaccttatggaactcattgatggaatatcactgggactaattttgctaaaaatagtaacacagtttgacaacacccaagtgggaaccttagctctttccttgactttcataagatcaacaatgccattggtcatggcttggaggaccattatggctgtgttgtttgtggtcacactcattcctttgtgcaggacaagctgtcttcaaaaacagtctcattgggtagaaataacagcactcatcctaggagcccaagctctgccagtgtacctaatgactcttatgaaaggagcctcaagaagatcttggcctcttaacgagggcataatggctgtgggtttggttagtctcttaggaagcgctcttttaaagaatgatgtccctttagctggcccaatggtggcaggaggcttacttctggcggcttacgtgatgagtggtagctcagcagatctgtcactagagaaggccgccaacgtgcagtgggatgaaatggcagacataacaggctcaagcccaatcatagaagtgaagcaggatgaagatggctctttctccatacgggacgtcgaggaaaccaatatgataacccttttggtgaaactggcactgataacagtgtcaggtctctaccccttggcaattccagtcacaatgaccttatggtacatgtggcaagtgaaaacacaaagatcaggagccctgtgggacgtcccctcacccgctgccactaaaaaagccgcactgtctgaaggagtgtacaggatcatgcaaagagggttattcgggaaaactcaggttggagtagggatacacatggaaggtgtatttcacacaatgtggcatgtaacaagaggatcagtgatctgccacgagactgggagattggagccatcttgggctgacgtcaggaatgacatgatatcatacggtgggggatggaggcttggagacaaatgggacaaagaagaagacgttcaggtcctcgccatagaaccaggaaaaaatcctaaacatgtccaaacgaaacctggccttttcaagaccctaactggagaaattggagcagtaacattagatttcaaacccggaacgtctggttctcccatcatcaacaggaaaggaaaagtcatcggactctatggaaatggagtagttaccaaatcaggtgattacgtcagtgccataacgcaagccgaaagaattggagagccagattatgaagtggatgaggacatttttcgaaagaaaagattaactataatggacttacaccccggagctggaaagacaaaaagaattcttccatcaatagtgagagaagccttaaaaaggaggctacgaactttgattttagctcccacgagagtggtggcggccgagatggaagaggccctacgtggactgccaatccgttatcagaccccagctgtgaaatcagaacacacaggaagagagattgtagacctcatgtgtcatgcaaccttcacaacaagacttttgtcatcaaccagggttccaaattacaaccttatagtgatggatgaagcacatttcaccgatccttctagtgtcgcggctagaggatacatctcgaccagggtggaaatgggagaggcagcagccatcttcatgaccgcaacccctcccggagcgacagatccctttccccagagcaacagcccaatagaagacatcgagagggaaattccggaaaggtcatggaacacagggttcgactggataacagactaccaagggaaaactgtgtggtttgttcccagcataaaagctggaaatgacattgcaaattgtttgagaaagtcgggaaagaaagttatccagttgagtaggaaaacctttgatacagagtatccaaaaacgaaactcacggactgggactttgtggtcactacagacatatctgaaatgggggccaattttagagccgggagagtgatagaccctagaagatgcctcaagccagttatcctaccagatgggccagagagagtcattttagcaggtcctattccagtgactccagcaagcgctgctcagagaagagggcgaataggaaggaacccagcacaagaagacgaccaatacgttttctccggagacccactaaaaaatgatgaagatcatgcccactggacagaagcaaagatgctgcttgacaatatctacaccccagaagggatcattccaacattgtttggtccggaaagggaaaaaacccaagccattgatggagagtttcgcctcagaggggaacaaaggaagacttttgtggaattaatgaggagaggagaccttccggtgtggctgagctataaggtagcttctgctggcatttcttacaaagatcgggaatggtgcttcacaggggaaagaaataaccaaattttagaagaaaacatggaggttgaaatttggactagagagggagaaaagaaaaagctaaggccaagatggttagatgcacgtgtatacgctgaccccatggctttgaaggatttcaaggagtttgccagtggaaggaagagtataactctcgacatcctaacagagattgccagtttgccaacttacctttcctctagggccaagctcgcccttgataacatagtcatgctccacacaacagaaagaggagggagggcctatcaacacgccctgaacgaacttccggagtcactggaaacactcatgcttgtagctttactaggtgctatgacagcaggcatcttcctgtttttcatgcaagggaaaggaatagggaaattgtcaatgggtttgataaccattgcggtggctagtggcttgctctgggtagcagaaattcaaccccagtggatagcggcctcaatcatactagagttttttctcatggtactgttgataccggaaccagaaaaacaaaggaccccacaagacaatcaattgatctacgtcatattgaccattctcaccatcattggtctaatagcagccaacgagatggggctgattgaaaaaacaaaaacggattttgggttttaccaggtaaaaacagaaaccaccatcctcgatgtggacttgagaccagcttcagcatggacgctctatgcagtagccaccacaattctgactcccatgctgagacacaccatagaaaacacgtcggccaacctatctctagcagccattgccaaccaggcagccgtcctaatggggcttggaaaaggatggccgctccacagaatggacctcggtgtgccgctgttagcaatgggatgctattctcaagtgaacccaacaaccttgacagcatccttagtcatgcttttcgtgcactatgcaataataggcccaggattgcaggcaaaagccacaagagaggcccagaaaaggacagctgctgggatcatgaaaaatcccacagtggacgggataacagtaatagatctagaaccaatatcctatgacccaaaatttgaaaagcaattagggcaggtcatgctactagtcttgtgtgctggacaactactcttgatgagaacaacatgggctttctgtgaagtcttgactttggccacaggaccaatcttgaccttgtgggagggcaacccgggaaggttttggaacacgaccatagccgtatccaccgccaacattttcaggggaagttacttggcgggagctggactggctttttcactcataaagaatgcacaaacccctaggaggggaactgggaccacaggagagacactgggagagaagtggaagagacagctaaactcattagacagaaaagagtttgaagagtataaaagaagtggaatactagaagtggacaggactgaagccaagtctgccctgaaagatgggtctaaaatcaagcatgcagtatcaagagggtccagtaagatcagatggattgttgagagagggatggtaaagccaaaagggaaagttgtagatcttggctgtgggagaggaggatggtcttattacatggcgacactcaagaacgtgactgaagtgaaagggtatacaaaaggaggtccaggacatgaagaaccgattcccatggctacttatggttggaatttggtcaaactccattcaggggttgacgtgttctacaaacccacagagcaagtggacaccctgctctgtgatattggggagtcatcttctaatccaacaatagaggaaggaagaacattaagagttttgaagatggtggagccatggctctcttcaaaacctgaattctgcatcaaagtccttaacccctacatgccaacagtcatagaagagctggagaaactgcagagaaaacatggtgggaaccttgtcagatgcccgctgtccaggaactccacccatgagatgtattgggtgtcaggagcgtcgggaaacattgtgagctctgtgaacacaacatcaaagatgttgttgaacaggttcacaacaaggcataggaaacccacttatgagaaggacgtagatcttggggcaggaacgagaagtgtctccactgaaacagaaaaaccagacatgacaatcattgggagaaggcttcagcgattgcaagaagagcacaaagaaacctggcattatgatcaggaaaacccatacagaacctgggcgtatcatggaagctatgaagctccttcgacaggctctgcatcctccatggtgaacggggtggtaaaactgctaacaaaaccctgggatgtgattccaatggtgactcagttagccatgacagatacaaccccttttgggcaacaaagagtgttcaaagagaaggtggataccagaacaccacaaccaaaacccggtacacgaatggttatgaccacgacagccaattggctgtgggccctccttggaaagaagaaaaatcccagactgtgcacaagggaagagttcatctcaaaagttagatcaaacgcagccataggcgcagtctttcaggaagaacagggatggacatcagccagtgaagctgtgaatgacagccggttttgggaactggttgacaaagaaagggccctacaccaggaagggaaatgtgaatcgtgtgtctataacatgatgggaaaacgtgagaaaaagttaggagagtttggcagagccaagggaagccgagcaatctggtacatgtggctgggagcgcggtttctggaatttgaagccctgggttttttgaatgaagatcactggtttggcagagaaaattcatggagtggagtggaaggggaaggtctgcacagattgggatatatcctggaggagatagacaagaaggatggagacctaatgtatgctgatgacacagcaggctgggacacaagaatcactgaggatgaccttcaaaatgaggaactgatcacggaacagatggctccccaccacaagatcctagccaaagccattttcaaactaacctatcaaaacaaagtggtgaaagtcctcagacccacaccgcggggagcggtgatggatatcatatccaggaaagaccaaagaggtagtggacaagttggaacatatggtttgaacacattcaccaacatggaagttcaactcatccgccaaatggaagctgaaggagtcatcacacaagatgacatgcagaacccaaaagggttgaaagaaagagttgagaaatggctgaaagagtgtggtgtcgacaggttaaagaggatggcaatcagtggagacgattgcgtggtgaagcccctagatgagaggtttggcacttccctcctcttcttgaacgacatgggaaaggtgaggaaagacattccgcagtgggaaccatctaagggatggaaaaactggcaagaggttcctttttgctcccaccactttcacaagatctttatgaaggatggccgctcactagttgttccatgtagaaaccaggatgaactgatagggagagccagaatctcgcagggagctggatggagcttaagagaaacagcctgcctgggcaaagcttacgcccagatgtggtcgcttatgtacttccacagaagggatctgcgtttagcctccatggccatatgctcagcagttccaacggaatggtttccaacaagcagaacaacatggtcaatccacgctcatcaccagtggatgaccactgaagatatgctcaaagtgtggaacagagtgtggatagaagacaaccctaatatgactgacaagactccagtccattcgtgggaagatataccttacctagggaaaagagaggatttgtggtgtggatccctgattggactttcttccagagccacctgggcgaagaacattcacacggccataacccaggtcaggaacctgatcggaaaagaggaatacgtggattacatgccagtaatgaaaagatacagtgctccttcagagagtgaaggagttctgtaattaccaacaacaaacaccaaaggctattgaagtcaggccacttgtgccacggtttgagcaaaccgtgctgcctgtagctccgccaataatgggaggcgtaataatccccagggaggccatgcgccacggaagctgtacgcgtggcatattggactagcggttagaggagacccctcccatcactgacaaaacgcagcaaaagggggcccaagactagaggttagaggagacccccccaacacaaaaacagcatattgacgctgggaaagaccagagatcctgctgtctctgcaacatcaatccaggcacagagcnnnnnnnnnnnnnnnnnnnnnnnnnnnnnnnnnnnnnnn

SEQ ID NO: 3 - DNA, 10645 bp, Dengue virus 3
  misc_feature (10644)..(10645): n is a, c, g, or t
agttgttagtctacgtggaccgacaagaacagtttcgactcggaagcttgcttaacgtagtactgacagttttttattagagagcagatctctgatgaacaaccaacggaaaaagacgggaaaaccgtctatcaatatgctgaaacgcgtgagaaaccgtgtgtcaactggatcacagttggcgaagagattctcaagaggactgctgaacggccaaggaccaatgaaattggttatggcgttcatagctttcctcagatttctagccattccaccgacagcaggagtcttggctagatggggaacctttaagaagtcgggggctattaaggtcctgagaggcttcaagaaggagatctcaaacatgctgagcattatcaacagacggaaaaagacatcgctctgtctcatgatgatgttaccagcaacacttgctttccacttgacttcacgagatggagagccgcgcatgattgtggggaagaatgaaagaggaaaatccctactttttaagacagcctctggaatcaacatgtgcacactcatagccatggatttgggagagatgtgtgatgacacggtcacctacaaatgccccctcattactgaagtggagcctgaagacattgactgctggtgcaaccttacatcgacatgggtgacctacggaacgtgcaatcaagctggagagcacagacgcgacaaaagatcggtggcgttagctccccatgtcggcatgggactggacacacgcacccaaacctggatgtcggctgaaggagcttggagacaggtcgagaaggtagagacatgggcctttaggcacccagggttcacaatactagccctatttcttgcccattacataggcacttccttgacccagaaagtggttattttcatactactaatgctggtcaccccatccatgacaatgagatgcgtgggagtaggaaacagagattttgtggaaggcctatcaggagctacgtgggttgacgtggtgctcgagcacggtgggtgtgtgactaccatggctaagaacaagcccacgctggatatagagctccagaagaccgaggccacccaactggcgaccctaaggaaactatgtattgagggaaaaattaccaacgtaacaaccgactcaaggtgccccacccaaggggaagcgattttacctgaggagcaggaccagaaccacgtgtgcaagcacacatacgtggacagaggctggggaaacggttgtggtttgtttggcaagggaagcctggtaacatgcgcgaaatttcaatgtttggaatcaatagagggaaaagtggtgcagcatgagaacctcaaatacaccgtcatcatcacagtgcacacaggagatcaacaccaggtgggaaatgaaacgcagggagtcacggctgagataacaccccaggcatcaaccgttgaagccatcttacctgaatatggaacccttgggctagaatgctcaccacggacaggtttagatttcaatgaaatgattttgttgacaatgaagaacagagcatggatggtacatagacaatggttttttgacctacctttaccatggacatcaggagctacaacagaaacaccaacctggaataagaaagagcttcttgtgacattcaaaaacgcacatgcaaaaaagcaagaagtagtggtccttggatcgcaagagggagcaatgcacacagcactgacaggagctacagagatccaaacctcaggaggcacaagtatttttgcggggcacttaaaatgtagactcaagatggacaaattggaactcaaggggatgagctatgcaatgtgcttgaatgcctttgtgttgaagaaagaagtctccgaaacgcaacatgggacaatactcatcaaggttgagtacaaaggggaagatgcaccttgcaagattcctttctccacggaggatggacaagggaaagcccacaatggcagactgatcacagctaacccagtggtgaccaagaaggaggagcctgtcaatattgaggcagaacctccttttggggaaagcaatatagtaattggaattggagacaaagccttgaaaattaactggtacaagaagggaagctcgattgggaagatgttcgaggccactgccagaggtgcaaggcgcatggccatcttgggagacacagcctgggactttggatcagtaggtggtgttttaaattcattaggaaaaatggtgcaccaaatatttggaagtgcttacacagccctatttagtggagtctcctggataatgaaaattggaataggtgtccttttaacctggatagggttgaattcaaaaaacactagtatgagctttagctgcattgtgataggaatcattacactctatctgggagccgtggtgcaagctgacatggggtgtgtcataaactggaaaggcaaagaactcaaatgtggaagtggaattttcgtcactaatgaggtccacacctggacagagcaatacaaatttcaagcagactcccccaaaagactggcgacagccattgcaggcgcttgggagaatggagtgtgcggaatcaggtcgacaaccagaatggagaacctcttgtggaagcaaatagccaatgaactgaactacatattatgggaaaacaacatcaaattaacggtagttgtgggtgatataattggggtcttagagcaagggaaaagaacactaacaccacaacccatggaactaaaatattcatggaaaacatggggaaaggcgaagatagtgacagctgaaacacaaaattcctctttcataatagatgggccaaacacaccagagtgtccaagtgcctcaagagcatggaatgtgtgggaggtggaagattacgggttcggagtcttcacaactaacatatggctgaaactccgagagatgtacacccaactatgtgaccacaggctaatgtcggcagccgttaaggatgagagggccgtacacgccgacatgggctattggatagaaagccaaaagaatggaagttggaagctagaaaaggcatccctcatagaggtaaaaacctgcacatggccaaaatcacacactctttggagcaatggtgtgctagagagtgacatgatcatcccaaagagtctggctggtcccatttcgcaacacaactacaggcccggataccacacccaaacggcaggaccctggcacttaggaaaattggagctggacttcaactattgtgaaggaacaacagttgtcatcacagaaaattgtgggacaagaggcccatcactgagaacaacaacagtgtcagggaagttgatacacgaatggtgttgccgctcgtgtacacttcctcccctgcgatacatgggagaagacggctgctggtatggcatggaaattagacccattaatgagaaagaagagaacatggtaaagtctttagtctcagcagggagtggaaaggtggataacttcacaatgggtgtcttgtgtttggcaatcctttttgaagaggtgatgagaggaaaatttgggaaaaagcacatgattgcaggggttctcttcacgtttgtactccttctctcagggcaaataacatggagagacatggcgcacacactcataatgattgggtccaacgcctctgacagaatgggaatgggcgtcacttacctagcattgattgcaacatttaaaattcagccatttttggctttgggattcttcctgaggaaactgacatctagagaaaatttattgttgggagttgggttggccatggcaacaacgttacaactgccagaggacattgaacaaatggcgaatggaatagctttagggctcatggctcttaaattaataacacaatttgaaacataccaactatggacggcattagtctccctaatgtgttcaaatacaattttcacgttgactgttgcctggagaacagccaccctgattttggccggaatttctcttttgccagtgtgccagtcttcgagcatgaggaaaacagattggctcccaatggctgtggcagctatgggagttccacccctaccactttttattttcagtttgaaagatacgctcaaaaggagaagctggccactgaatgagggggtgatggctgttggacttgtgagtattctagctagttctctccttaggaatgacgtgcccatggctggaccattagtggctgggggcttgctgatagcgtgctacgtcataactggcacgtcagcagacctcactgtagaaaaagcagcagatgtgacatgggaggaagaggctgagcaaacaggagtgtcccacaatttaatgatcacagttgatgacgatggaacaatgagaataaaagatgatgagactgagaacatcttaacagtgcttttgaaaacagcattactaatagtgtcaggcatttttccatactccatacccgcaacactgttggtctggcacacttggcaaaagcaaacccaaagatccggtgtcctatgggacgttcccagccccccagagacacagaaagcagaactggaagaaggggtttataggatcaagcagcaaggaatttttgggaaaacccaagtgggggttggagtacaaaaagaaggagttttccacaccatgtggcacgtcacaagaggagcagtgttgacacacaatgggaaaagactggaaccaaactgggctagcgtgaaaaaagatctgatttcatacggaggaggatggaaattgagtgcacaatggcaaaaaggagaggaggtgcaggttattgccgtagagcctgggaagaacccaaagaactttcaaaccatgccaggcattttccagacaacaacaggggagataggagcgattgcactggacttcaagcctggaacttcaggatctcccatcataaacagagagggaaaggtactgggattgtatggcaatggagtggtcacaaagaatggtggctatgtcagtggaatagcacaaacaaatgcagaaccagacggaccgacaccagagttggaagaagagatgttcaaaaagcgaaatctaaccataatggatctccatcccgggtcaggaaagacgcggaaatatcttccagctattgttagagaggcaatcaagagacgcttaaggactctaattttggcaccaacaagggtagttgcagctgagatggaagaagcattgaaagggctcccaataaggtatcaaacaactgcaacaaaatctgaacacacagggagagagattgttgatctaatgtgccacgcaacgttcacaatgcgtttgctgtcaccagtcagggttccaaactacaacttgataataatggatgaggctcatttcacagacccagccagtatagcggctagagggtacatatcaactcgtgtaggaatgggagaggcagccgcaattttcatgacagccacaccccctggaacagctgatgcctttcctcagagcaacgctccaattcaagatgaagaaagagacataccagaacgctcatggaattcaggcaatgaatggattaccgactttgccgggaagacggtgtggtttgtccctagcatcaaagctggaaatgacatagcaaactgcttgcggaaaaatggaaaaaaggtcattcaacttagtaggaagacttttgacacagaatatcaaaagactaaactaaatgattgggactttgtggtgacaacagacatttcagaaatgggagccaatttcaaagcagacagagtgatcgacccaagaagatgtctcaagccagtgattttgacagacggacccgagcgcgtgatcctggcgggaccaatgccagtcaccgtagcgagcgctgcgcaaaggagagggagagttggcaggaacccacaaaaagaaaatgaccaatacatattcatgggccagcccctcaataatgatgaagaccatgctcactggacagaagcaaaaatgctgctagacaacatcaacacaccagaagggatcataccagctctctttgaaccagaaagggagaagtcagccgccatagacggcgaataccgcctgaagggtgagtccaggaagaccttcgtggaactcatgaggaggggtgacctcccagtttggctagcccataaagtagcatcagaagggatcaaatatacagatagaaagtggtgttttgatggagaacgcaacaatcaaattttagaggagaatatggatgtggaaatctggacaaaggaaggagaaaagaaaaaattgagacctaggtggcttgatgcccgcacttattcagatcccttagcgctcaaggaattcaaggactttgcggctggtagaaagtcaattgcccttgatcttgtgacagaaataggaagagtgccttcacacttagctcacagaacgagaaacgccctggacaatctggtgatgttgcacacgtcagaacatggcgggagggcctacaggcatgcagtggaggaactaccagaaacaatggaaacactcttactcctgggactcatgatcctgttaacaggtggagcaatgcttttcttgatatcaggtaaagggattggaaagacttcaataggactcatttgtgtagctgcttccagcggtatgttatggatggctgatgtcccactccaatggatcgcgtctgccatagtcctggagttttttatgatggtgttacttataccagaaccagaaaagcagagaactccccaagacaatcaactcgcatatgtcgtgataggcatactcacactggctgcaatagtagcagccaatgaaatgggactgttggaaaccacaaagagagatttaggaatgtccaaagaaccaggtgttgtttctccaaccagctatttggatgtggacttgcacccagcatcagcctggacattgtacgctgtggccacaacagtaataacaccaatgttgagacataccatagagaattccacagcaaatgtgtccctggcagctatagccaaccaggcagtggtcctgatgggtttagacaaaggatggccgatatcgaaaatggacttaggcgtgccactattggcactgggttgttattcacaagtgaacccactaactctcacagcggcagttctcctgctagccacgcattatgctattataggtccaggattgcaggcaaaagccactcgtgaagctcaaaaaaggacagctgctggaataatgaagaatccaacggtggatgggataatgacaatagacctagatcctgtaatatacgatccaaaatttgaaaagcaactaggacaggttatgctcctggttctgtgtgcagttcaacttttgttaatgagaacatcatgggctttttgtgaagctctaaccctagccacaggaccaataacaacactctgggaaggatcacctgggaagttctggaacaccacgatagctgtttccatggcgaacatctttagagggagctatttagcaggagctgggcttgctttttctatcatgaaatcagttggaacaggaaagagagggacagggtcacagggtgaaaccttgggagaaaagtggaaaaagaaattgaatcaattaccccggaaagagtttgacctttacaagaaatccggaatcactgaagtggatagaacagaagccaaagaagggttgaaaagaggagaaataacacaccatgccgtgtccagaggcagcgcaaaacttcaatggttcgtggagagaaacatggtcatccccgaaggaagagtcatagacttaggctgtggaagaggaggctggtcatattattgtgcaggactgaaaaaagttacagaagtgcgaggatacacaaaaggcggcccaggacatgaagaaccagtacctatgtctacatacggatggaacatagtcaagttaatgagtggaaaggatgtgttttatcttccacctgaaaagtgtgatactctattgtgtgacattggagaatcttcaccaagcccaacagtggaagaaagcagaaccataagagtcttgaagatggttgaaccatggctaagaaataaccagttttgcattaaagtattgaacccttacatgccaactgtgattgagcacctagaaagactacaaaggaaacatggaggaatgcttgtgagaaatccactctcacgaaactccacgcacgaaatgtactggatatctaatggcacaggcaatatcgtttcttcagtcaacatggtatccagattgctacttaacagattcacaatgacacataggagacccaccatagagaaagatgtggatttaggagcggggacccgacatgtcaatgcggaaccagaaacacccaacatggatgtcattggggaaagaataagaaggatcaaggaggagcatagttcaacatggcactatgatgatgaaaatccttataaaacgtgggcttaccatggatcctatgaagttaaggccacaggctcagcctcctccatgataaatggagtcgtgaaactcctcacgaaaccatgggatgtggtgcccatggtgacacagatggcaatgacggatacaaccccattcggccagcaaagggtttttaaagagaaagtggacaccaggacacccagacctatgccaggaacaagaaaggttatggagatcacagcggaatggctttggagaaccctgggaaggaacaaaagacccagattatgtacgagagaggagttcacaaaaaaggtcagaaccaacgcagctatgggcgccgtttttacagaggagaaccaatgggacagtgctagagctgctgttgaggatgaagaattctggaaactcgtggacagagaacgtgaactccacaaattgggcaagtgtggaagctgcgtttacaacatgatgggcaagagagagaagaaacttggagagtttggcaaagcaaaaggcagtagagccatatggtacatgtggttgggagccagataccttgagttcgaagcactcggattcttaaatgaagaccattggttctcgcgtgaaaactcttacagtggagtagaaggagaaggactgcacaagctgggatacatcttaagagacatttccaagatacccggaggagctatgtatgctgatgacacagctggttgggacacaagaataacagaagatgacctgcacaatgaggaaaaaatcacacagcaaatggaccctgaacacaggcagttagcaaacgctatattcaagctcacataccaaaacaaagtggtcaaagttcaacgaccaactccaaagggcacggtaatggacatcatatctaggaaagaccaaagaggcagtggacaggtgggaacttatggtctgaatacattcaccaacatggaagcccagttaatcagacaaatggaaggagaaggtgtgttgtcgaaggcagacctcgagaaccctcatctgctagagaagaaagttacacaatggttggaaacaaaaggagtggagaggttaaaaagaatggccatcagcggggatgattgcgtggtgaaaccaattgatgacaggttcgccaatgccctgcttgccctgaatgacatgggaaaagttaggaaggacatacctcaatggcagccatcaaagggatggcatgattggcaacaggtccctttctgctcccaccactttcatgaattgatcatgaaagatggaagaaagttggtagttccctgcagacctcaggatgaattaatcgggagagcgagaatctctcaaggagcaggatggagccttagagaaactgcatgcctagggaaagcctacgcccaaatgtggactctcatgtactttcacagaagagatcttagactagcatccaacgccatatgttcagcagtaccagtccattgggtccccacaagcagaacgacgtggtctattcatgctcaccatcagtggatgactacagaagacatgcttactgtttggaacagggtgtggatagaggataatccatggatggaagacaaaactccagtcaaaacctgggaagatgttccatatctagggaagagagaagaccaatggtgcggatcactcattggtctcacttccagagcaacctgggcccagaacatacttacggcaatccaacaggtgagaagccttataggcaatgaagagtttctggactacatgccttcgatgaagagattcaggaaggaggaggagtcagagggagccatttggtaaacgtaggaagtgaaaaagaggcaaactgtcaggccaccttaagccacagtacggaagaagctgtgcagcctgtgagccccgtccaaggacgttaaaagaagaagtcaggcccaaaagccacggtttgagcaaaccgtgctgcctgtggctccgtcgtggggacgtaaaacctgggaggctgcgactagcggttagaggagacccctcccgtgacacaacgcagcagcggggcccaagactagaggttagaggagaccccccgcaaataaaaacagcatattgacgctgggagagaccagagatcctgctgtctcctcagcatcattccaggcacagaacgccagaaaatggaatggtgctgttgaatcaacaggttnn

SEQ ID NO: 4 - DNA, 10618 bp, Dengue virus 4
  misc_feature (1)..(16): n is a, c, g, or t
  misc_feature (10579)..(10618): n is a, c, g, or t
nnnnnnnnnnnnnnnnggaccgacaaggacagttccaaatcggaagcttgcttaacacagttctaacagtttgtttgaatagagagcagatctctggaaaaatgaaccaacgaaaaaaggtggttagaccacctttcaatatgctgaaacgcgagagaaaccgcgtatcaacccctcaagggttggtgaagagattctcaaccggacttttttctgggaaaggacccttacggatggtgctagcattcatcacgtttttgcgagtcctttccatcccaccaacagcagggattctgaagagatggggacagttgaagaaaaataaggccatcaagatactgattggattcaggaaggagataggccgcatgctgaacatcttgaacgggagaaaaaggtcaacgataacattgctgtgcttgattcccaccgtaatggcgttttccctcagcacaagagatggcgaacccctcatgatagtggcaaaacatgaaagggggagacctctcttgtttaagacaacagaggggatcaacaaatgcactctcattgccatggacttgggtgaaatgtgtgaggacactgtcacgtataaatgccccctactggtcaataccgaacctgaagacattgattgctggtgcaacctcacgtctacctgggtcatgtatgggacatgcacccagagcggagaacggagacgagagaagcgctcagtagctttaacaccacattcaggaatgggattggaaacaagagctgagacatggatgtcatcggaaggggcttggaagcatgctcagagagtagagagctggatactcagaaacccaggattcgcgctcttggcaggatttatggcttatatgattgggcaaacaggaatccagcgaactgtcttctttgtcctaatgatgctggtcgccccatcctacggaatgcgatgcgtaggagtaggaaacagagactttgtggaaggagtctcaggtggagcatgggtcgacctggtgctagaacatggaggatgcgtcacaaccatggcccagggaaaaccaaccttggattttgaactgactaagacaacagccaaggaagtggctctgttaagaacctattgcattgaagcctcaatatcaaacataactacggcaacaagatgtccaacgcaaggagagccttatctgaaagaggaacaggaccaacagtacatttgccggagagatgtggtagacagagggtggggcaatggctgtggcttgtttggaaaaggaggagttgtgacatgtgcgaagttttcatgttcggggaagataacaggcaatttggtccaaattgagaaccttgaatacacagtggttgtaacagtccacaatggagacacccatgcagtaggaaatgacacatccaatcatggagttacagccatgataactcccaggtcaccatcggtggaagtcaaattgccggactatggagaactaacactcgattgtgaacccaggtctggaattgactttaatgagatgattctgatgaaaatgaaaaagaaaacatggctcgtgcataagcaatggtttttggatctgcctcttccatggacagcaggagcagacacatcagaggttcactggaattacaaagagagaatggtgacatttaaggttcctcatgccaagagacaggatgtgacagtgctgggatctcaggaaggagccatgcattctgccctcgctggagccacagaagtggactccggtgatggaaatcacatgtttgcaggacatcttaagtgcaaagtccgtatggagaaattgagaatcaagggaatgtcatacacgatgtgttcaggaaagttttcaattgacaaagagatggcagaaacacagcatgggacaacagtggtgaaagtcaagtatgaaggtgctggagctccgtgtaaagtccccatagagataagagatgtaaacaaggaaaaagtggttgggcgtatcatctcatccacccctttggctgagaataccaacagtgtaaccaacatagaattagaacccccctttggggacagctacatagtgataggtgttggaaacagcgcattaacactccattggttcaggaaagggagttccattggcaagatgtttgagtccacatacagaggtgcaaaacgaatggccattctaggtgaaacagcttgggattttggttccgttggtggactgttcacatcattgggaaaggctgtgcaccaggtttttggaagtgtgtatacaaccatgtttggaggagtctcatggatgattagaatcctaattgggttcttagtgttgtggattggcacgaactcgaggaacacttcaatggctatgacgtgcatagctgttggaggaatcactctgtttctgggcttcacagttcaagcagacatgggttgtgtggcgtcatggagtgggaaagaattgaagtgtggaagcggaatttttgtggttgacaacgtgcacacttggacagaacagtacaaatttcaaccagagtccccagcgagactagcgtctgcaatattaaatgcccacaaagatggggtctgtggaattagatcaaccacgaggctggaaaatgtcatgtggaagcaaataaccaacgagctaaactatgttctctgggaaggaggacatgacctcactgtagtggctggggatgtgaagggggtgttgaccaaaggcaagagagcactcacacccccagtgagtgatctgaaatattcatggaagacatggggaaaagcaaaaatcttcaccccagaagcaagaaatagcacatttttaatagacggaccagacacctctgaatgccccaatgaacgaagagcatggaactctcttgaggtggaagactatggatttggcatgttcacgaccaacatatggatgaaattccgagaaggaagttcagaagtgtgtgaccacaggttaatgtcagctgcaattaaagatcagaaagctgtgcatgctgacatgggttattggatagagagctcaaaaaaccagacctggcagatagagaaagcatctcttattgaagtgaaaacatgtctgtggcccaagacccacacactgtggagcaatggagtgctggaaagccagatgctcattccaaaatcatatgcgggccctttttcacagcacaattaccgccagggctatgccacgcaaaccgtgggcccatggcacttaggcaaattagagatagactttggagaatgccccggaacaacagtcacaattcaggaggattgtgaccatagaggcccatctttgaggaccaccactgcatctggaaaactagtcacgcaatggtgctgccgctcctgcacgatgcctcccttaaggttcttgggagaagatgggtgctggtatgggatggagattaggcccttgagtgaaaaagaagagaacatggtcaaatcacaggtgacggccggacagggcacatcagaaactttttctatgggtctgttgtgcctgaccttgtttgtggaagaatgcttgaggagaagagtcactaggaaacacatgatattagttgtggtgatcactctttgtgctatcatcctgggaggcctcacatggatggacttactacgagccctcatcatgttgggggacactatgtctggtagaataggaggacagatccacctagccatcatggcagtgttcaagatgtcaccaggatacgtgctgggtgtgtttttaaggaaactcacttcaagagagacagcactaatggtaataggaatggccatgacaacggtgctttcaattccacatgaccttatggaactcattgatggaatatcactgggactaattttgctaaaaatagtaacacagtttgacaacacccaagtgggaaccttagctctttccttgactttcataagatcaacaatgccattggtcatggcttggaggaccattatggctgtgttgtttgtggtcacactcattcctttgtgcaggacaagctgtcttcaaaaacagtctcattgggtagaaataacagcactcatcctaggagcccaagctctgccagtgtacctaatgactcttatgaaaggagcctcaagaagatcttggcctcttaacgagggcataatggctgtgggtttggttagtctcttaggaagcgctcttttaaagaatgatgtccctttagctggcccaatggtggcaggaggcttacttctggcggcttacgtgatgagtggtagctcagcagatctgtcactagagaaggccgccaacgtgcagtgggatgaaatggcagacataacaggctcaagcccaatcatagaagtgaagcaggatgaagatggctctttctccatacgggacgtcgaggaaaccaatatgataacccttttggtgaaactggcactgataacagtgtcaggtctctaccccttggcaattccagtcacaatgaccttatggtacatgtggcaagtgaaaacacaaagatcaggagccctgtgggacgtcccctcacccgctgccactaaaaaagccgcactgtctgaaggagtgtacaggatcatgcaaagagggttattcgggaaaactcaggttggagtagggatacacatggaaggtgtatttcacacaatgtggcatgtaacaagaggatcagtgatctgccacgagactgggagattggagccatcttgggctgacgtcaggaatgacatgatatcatacggtgggggatggaggcttggagacaaatgggacaaagaagaagacgttcaggtcctcgccatagaaccaggaaaaaatcctaaacatgtccaaacgaaacctggccttttcaagaccctaactggagaaattggagcagtaacattagatttcaaacccggaacgtctggttctcccatcatcaacaggaaaggaaaagtcatcggactctatggaaatggagtagttaccaaatcaggtgattacgtcagtgccataacgcaagccgaaagaattggagagccagattatgaagtggatgaggacatttttcgaaagaaaagattaactataatggacttacaccccggagctggaaagacaaaaagaattcttccatcaatagtgagagaagccttaaaaaggaggctacgaactttgattttagctcccacgagagtggtggcggccgagatggaagaggccctacgtggactgccaatccgttatcagaccccagctgtgaaatcagaacacacaggaagagagattgtagacctcatgtgtcatgcaaccttcacaacaagacttttgtcatcaaccagggttccaaattacaaccttatagtgatggatgaagcacatttcaccgatccttctagtgtcgcggctagaggatacatctcgaccagggtggaaatgggagaggcagcagccatcttcatgaccgcaacccctcccggagcgacagatccctttccccagagcaacagcccaatagaagacatcgagagggaaattccggaaaggtcatggaacacagggttcgactggataacagactaccaagggaaaactgtgtggtttgttcccagcataaaagctggaaatgacattgcaaattgtttgagaaagtcgggaaagaaagttatccagttgagtaggaaaacctttgatacagagtatccaaaaacgaaactcacggactgggactttgtggtcactacagacatatctgaaatgggggccaattttagagccgggagagtgatagaccctagaagatgcctcaagccagttatcctaccagatgggccagagagagtcattttagcaggtcctattccagtgactccagcaagcgctgctcagagaagagggcgaataggaaggaacccagcacaagaagacgaccaatacgttttctccggagacccactaaaaaatgatgaagatcatgcccactggacagaagcaaagatgctgcttgacaatatctacaccccagaagggatcattccaacattgtttggtccggaaagggaaaaaacccaagccattgatggagagtttcgcctcagaggggaacaaaggaagacttttgtggaattaatgaggagaggagaccttccggtgtggctgagctataaggtagcttctgctggcatttcttacaaagatcgggaatggtgcttcacaggggaaagaaataaccaaattttagaagaaaacatggaggttgaaatttggactagagagggagaaaagaaaaagctaaggccaagatggttagatgcacgtgtatacgctgaccccatggctttgaaggatttcaaggagtttgccagtggaaggaagagtataactctcgacatcctaacagagattgccagtttgccaacttacctttcctctagggccaagctcgcccttgataacatagtcatgctccacacaacagaaagaggagggagggcctatcaacacgccctgaacgaacttccggagtcactggaaacactcatgcttgtagctttactaggtgctatgacagcaggcatcttcctgtttttcatgcaagggaaaggaatagggaaattgtcaatgggtttgataaccattgcggtggctagtggcttgctctgggtagcagaaattcaaccccagtggatagcggcctcaatcatactagagttttttctcatggtactgttgataccggaaccagaaaaacaaaggaccccacaagacaatcaattgatctacgtcatattgaccattctcaccatcattggtctaatagcagccaacgagatggggctgattgaaaaaacaaaaacggattttgggttttaccaggtaaaaacagaaaccaccatcctcgatgtggacttgagaccagcttcagcatggacgctctatgcagtagccaccacaattctgactcccatgctgagacacaccatagaaaacacgtcggccaacctatctctagcagccattgccaaccaggcagccgtcctaatggggcttggaaaaggatggccgctccacagaatggacctcggtgtgccgctgttagcaatgggatgctattctcaagtgaacccaataaccttgacagcatccttagtcatgcttttcgtccattatgcaataataggcccaggattgcaggcaaaagccacaagagaggcccagaaaaggacagctgctgggatcatgaaaaatcccacagtggacgggataacagtaatagatctagaaccaatatcctatgacccaaaatttgaaaagcaattagggcaggtcatgctactagtcttgtgtgctggacaactactcttgatgagaacaacatgggctttctgtgaagtcttgactttggccacaggaccaatcttgaccttgtgggagggcaacccgggaaggttttggaacacgaccatagccgtatccaccgccaacattttcaggggaagttacttggcgggagctggactggctttttcactcataaagaatgcacaaacccctaggaggggaactgggaccacaggagagacactgggagagaagtggaagagacagctaaactcattagacagaaaagagtttgaagagtataaaagaagtggaatactagaagtggacaggactgaagccaagtctgccctgaaagatgggtctaaaatcaagcatgcagtatcaagagggtccagtaagatcagatggattgttgagagagggatggtaaagccaaaagggaaagttgtagatcttggctgtgggagaggaggatggtcttattacatggcgacactcaagaacgtgactgaagtgaaagggtatacaaaaggaggtccaggacatgaagaaccgattcccatggctacttatggttggaatttggtcaaactccattcaggggttgacgtgttctacaaacccacagagcaagtggacaccctgctctgtgatattggggagtcatcttctaatccaacaatagaggaaggaagaacattaagagttttgaagatggtggagccatggctctcttcaaaacctgaattctgcatcaaagtccttaacccctacatgccaacagtcatagaagagctggagaaactgcagagaaaacatggtgggaaccttgtcagatgcccgctgtccaggaactccacccatgagatgtattgggtgtcaggagcgtcgggaaacattgtgagctctgtgaacacaacatcaaagatgttgttgaacaggttcacaacaaggcataggagacctacttatgagaaggacgtagatcttggggcaggaacgagaagtgtctccactgaaacagaaaaaccagacatgacaatcattgggagaaggcttcagcgattgcaagaagagcacaaagaaacctggcattatgatcaggaaaacccatacagaacctgggcgtatcatggaagctatgaagctccttcgacaggctctgcatcctccatggtgaacggggtggtaaaactgctaacaaaaccctgggatgtgattccaatggtgactcagttagccatgacagatacaaccccttttgggcaacaaagagtgttcaaagagaaggtggataccagaacaccacaaccaaaacccggtacacgaatggttatgaccacgacagccaattggctgtgggccctccttggaaagaagaaaaatcccagactgtgcacaagggaagagttcatctcaaaagttagatcaaacgcagccataggcgcagtctttcaggaagaacagggatggacatcagccagtgaagctgtgaatgacagccggttttgggaactggttgacaaagaaagggccctacaccaggaagggaaatgtgaatcgtgtgtctataacatgatgggaaaacgtgagaaaaagttaggagagtttggcagagccaagggaagccgagcaatctggtacatgtggctgggagcgcggtttctggaatttgaagccctgggttttttgaatgaagatcactggtttggcagagaaaattcatggagtggagtggaaggggaaggtctgcacagattgggatatatcctggaggagatagacaagaaggatggagacctaatgtatgctgatgacacagcaggctgggacacaagaatcactgaggatgaccttcaaaatgaggaactgatcacggaacagatggctccccaccacaagatcctagccaaagccattttcaaactaacctatcaaaacaaagtggtgaaagtcctcagacccacaccgcggggagcggtgatggatatcatatccaggaaagaccaaagaggtagtggacaagttggaacatatggtttgaacacattcaccaacatggaagttcaactcatccgccaaatggaagctgaaggagtcatcacacaagatgacatgcagaacccaaaagggttgaaagaaagagttgagaaatggctgaaagagtgtggtgtcgacaggttaaagaggatggcaatcagtggagacgattgcgtggtgaagcccctagatgagaggtttggcacttccctcctcttcttgaacgacatgggaaaggtgaggaaagacattccgcagtgggaaccatctaagggatggaaaaactggcaagaggttcctttttgctcccaccactttcacaagatctttatgaaggatggccgctcactagttgttccatgtagaaaccaggatgaactgatagggagagccagaatctcgcagggagctggatggagcttaagagaaacagcctgcctgggcaaagcttacgcccagatgtggtcgcttatgtacttccacagaagggatctgcgtttagcctccatggccatatgctcagcagttccaacggaatggtttccaacaagcagaacaacatggtcaatccacgctcatcaccagtggatgaccactgaagatatgctcaaagtgtggaacagagtgtggatagaagacaaccctaatatgactgacaagactccagtccattcgtgggaagatataccttacctagggaaaagagaggatttgtggtgtggatccctgattggactttcttccagagccacctgggcgaagaacattcacacggccataacccaggtcaggaacctgatcggaaaagaggaatacgtggattacatgccagtaatgaaaagatacagtgctccttcagagagtgaaggagttctgtaattaccaacaacaaacaccaaaggctattgaagtcaggccacttgtgccacggtttgagcaaaccgtgctgcctgtagctccgccaataatgggaggcgtaataatccccagggaggccatgcgccacggaagctgtacgcgtggcatattggactagcggttagaggagacccctcccatcactgacaaaacgcagcaaaagggggcccaagactagaggttagaggagacccccccaacacaaaaacagcatattgacgctgggaaagaccagagatcctgctgtctctgcaacatcaatccaggcacagagnnnnnnnnnnnnnnnnnnnnnnnnnnnnnnnnnnnnnnnn